European Patent Specification EP 3 018 205 B1, published March 5, 2025. Title: Root-knot nematode resistance marker of Solanum Lycopersicum, root-knot nematode resistance Solanum Lycopersicum, production method of root-knot nematode resistance Solanum Lycopersicum and screening method of root-knot nematode resistance Solanum Lycopersicum. Applicant: Takii & Co.,Ltd. The sequence listing filed with the application follows.

SEQUENCE LISTING (34 sequences)

SEQ ID NO: 1 - DNA, 101 bp, Solanum Lycopersicum
atgctttcttcaactccgacttctgtaataccagaatttatcgtggtggaggttccgggaactgcatggaggaaggttttaaccccagttcaatccatata

SEQ ID NO: 2 - DNA, 116 bp, Solanum Lycopersicum
cgtacagctgcatagctttctcaatctccttattcctagacaactcttctattagaacgccataaacagaaatgtccagcacaaaacccaatttcttcattttatccaacagttgc

SEQ ID NO: 3 - DNA, 101 bp, Solanum Lycopersicum
ttggagatcgggtcagcttgtgtgccacagaggagagggtttgaagacgaggcaagaatctggcatcttatgcaacaaaaacctttagatcaagggaaatt

SEQ ID NO: 4 - DNA, 101 bp, Solanum Lycopersicum
cgaaatgctcttttttcctttacaccatgtgactgattatagtcttactttaatgaataagcaactgaatacaaaaattatcacctctatatagatacagt

SEQ ID NO: 5 - DNA, 101 bp, Solanum Lycopersicum
tctccggcgaccggagaatcctacgcctgtaaatctatcgataaaaaccttctcattgattccaccgaccgtgagtgtctcgataaagaacccaaaattct

SEQ ID NO: 6 - DNA, 101 bp, Solanum Lycopersicum
agtggctttatgctctactagggagcacgggcgctgcaatatttggttcctttaatcccctcttggcctatgtcattgcattgattgtaacagcatattac

SEQ ID NO: 7 - DNA, 99 bp, Solanum Lycopersicum
ttgccagcagagcggtccacgttggcgaggcggtactcgtgcataatccaattggtttttatacctctgggtgcttttccggcatagaacacaagtgcc

SEQ ID NO: 8 - DNA, 101 bp, Solanum Lycopersicum
tggtgaagaagcttgatcgagttggtgcccgccttgttagtagcaattcatgatgatcgatggatcaatcaatcaatcaactatgcctcaattccaaacga

SEQ ID NO: 9 - DNA, 132 bp, Solanum Lycopersicum
taacaaaaggcaaattaatgggaacaagggactgacatcaggagcttccaaagtcatattttaggtcttaggcaaagaaggtgataatttaactgtatgatccccatcaggccttcaaagacattgctaaaa

SEQ ID NO: 10 - DNA, 105 bp, Solanum Lycopersicum
agctaaagatatggtggaaaagtgtagaggcttacctcttgcaatcgttgtattgagcggactactttcacataaaagggggctagaccaatggcaaaaagtgaa

SEQ ID NO: 11 - DNA, 106 bp, Solanum Lycopersicum
gctgtgcaatgacttttgcattcaggtcctggaacttggggcattgacagtgctgatgaagatgatgaaatctcacaccacggaagaagctgtaaaagcattattt

SEQ ID NO: 12 - DNA, 116 bp, Solanum Lycopersicum
tattcatgaacaaaaaacagtgagaaaaatgtgtcatacgactcaaactcattcagccaaagacgtctatcaatattgtccagttattaataataactttttttttttctgtttgc

SEQ ID NO: 13 - DNA, 31 bp, Solanum Lycopersicum
agggtttgaagacgaggcaagaatctggcat

SEQ ID NO: 14 - DNA, 31 bp, Solanum Lycopersicum
attatagtcttactttaatgaataagcaact

SEQ ID NO: 15 - DNA, 41 bp, Solanum Lycopersicum
ccagaatttatcgtggtggaggttcttggaactgcatggag

SEQ ID NO: 16 - DNA, 79 bp, Solanum Lycopersicum
agaatcctacgcctgtaaatctatcgacaaaaaccttctcattgattccaccgaccgtgagtgtctcgataaagaaccc

SEQ ID NO: 17 - DNA, 31 bp, Solanum Lycopersicum
gttagtagcaattcatgatgatcgatggatc

SEQ ID NO: 18 - DNA, 32 bp, Solanum Lycopersicum
aagaaggtgaatatttaactgtatgatcccca

SEQ ID NO: 19 - DNA, 122 bp, Solanum Lycopersicum
ggtaaggatagctaaagatatggtggaaaagtgtagaggcttacctcttgcaatcgttgtattgagcggactactttcacataaaagggggctagaccaatggcaaaaagtgaaagatcact

SEQ ID NO: 20 - DNA, 31 bp, Solanum Lycopersicum
gcaatatttggttcctttaatcccctcttgg

SEQ ID NO: 21 - DNA, 31 bp, Solanum Lycopersicum
ctcaaactcattcagccaaagacgtctatca

SEQ ID NO: 22 - DNA, 41 bp, Solanum Lycopersicum
ctagacaactcttctattagaacaccataaacagaaatgtc

SEQ ID NO: 23 - DNA, 31 bp, Solanum Lycopersicum
ggcattgacagtgctgatgaagatgatgaaa

SEQ ID NO: 24 - DNA, 51 bp, Solanum Lycopersicum
gaaaagcacctagaggaataaaaaccaattggattatgcacgagtaccgcc

SEQ ID NO: 25 - DNA, 84 bp, Solanum Lycopersicum
aatctccttattcctagacaactcttctattagaacaccataaacagaaatgtccagcacaaaacccaatttcttcattttatc

SEQ ID NO: 26 - DNA, 141 bp, Solanum Lycopersicum
gctattgtattgacgctgtgcaatgacttttgcattcaggtcctggaacttggggcattgacagtgctgatgaagatgatgaaatctcacaccacagaagaagctgtaaaagcattatttgctatttcagcactaataaga

SEQ ID NO: 27 - DNA, 75 bp, Solanum Lycopersicum
agaaggcacttgtgttctatgccggaaaagcacctagaggaataaaaaccaattggattatgcacgagtaccgcc

SEQ ID NO: 28 - DNA, 61 bp, Solanum Lycopersicum
acagaggagagggtttgaagacgaggcaagaatctggcatcttatgcaacaaaaaccttta

SEQ ID NO: 29 - DNA, 88 bp, Solanum Lycopersicum
tcttcaactccgacttctgtaataccagaatttatcgtggtggaggttcttggaactgcatggaggaaggttttaaccccagttcaat

SEQ ID NO: 30 - DNA, 60 bp, Solanum Lycopersicum
gcgctgcaatatttggttcctttaatcccctcttggcctatgtcattgcattgattgtaa

SEQ ID NO: 31 - DNA, 82 bp, Solanum Lycopersicum
tgaagaagcttgatcgagttggtgcccgccttgttagtagcaattcatgatgatcgatggatcaatcaatcaatcaactatg

SEQ ID NO: 32 - DNA, 92 bp, Solanum Lycopersicum
aatgggaacaagggactgacatcaggagcttccaaagaaggtgaatatttaactgtatgatccccatcaggccttcaaagacattgctaaaa

SEQ ID NO: 33 - DNA, 61 bp, Solanum Lycopersicum
cctttacaccatgtgactgattatagtcttactttaatgaataagcaactgaatacaaaaa

SEQ ID NO: 34 - DNA, 105 bp, Solanum Lycopersicum
ttttattcatgaacaaaaaacagtgagaaaaatgtgtcatacgactcaaactcattcagccaaagacgtctatcaatattgtccagttattaataataacttttt